European Patent Specification EP 3 635 140 B1, published May 31, 2023. Title: DETECTING BABESIA SPECIES NUCLEIC ACID IN A SAMPLE. Applicant: GEN-PROBE INCORPORATED BRES, Vanessa SELF, Deanna LINNEN, Jeffrey M. Application TBA. The sequence listing filed with the application follows.

SEQUENCE LISTING (101 sequences)

SEQ ID NO: 1 - DNA, 52 bp, Artificial Sequence
  Synthetic Oligonucleotide
  promoter (1)..(27)
aatttaatacgactcactatagggagattcacctctgacagttaaatacgaa

SEQ ID NO: 2 - DNA, 25 bp, Artificial Sequence
  Synthetic Oligonucleotide
ttcacctctgacagttaaatacgaa

SEQ ID NO: 3 - DNA, 51 bp, Artificial Sequence
  Synthetic Oligonucleotide
  promoter (1)..(27)
aatttaatacgactcactatagggagaacagttaaatacgaatgcccccaa

SEQ ID NO: 4 - DNA, 24 bp, Artificial Sequence
  Synthetic Oligonucleotide
acagttaaatacgaatgcccccaa

SEQ ID NO: 5 - DNA, 49 bp, Artificial Sequence
  Synthetic Oligonucleotide
  promoter (1)..(27)
aatttaatacgactcactatagggagattcacctctgacagttaaatac

SEQ ID NO: 6 - DNA, 22 bp, Artificial Sequence
  Synthetic Oligonucleotide
ttcacctctgacagttaaatac

SEQ ID NO: 7 - DNA, 57 bp, Artificial Sequence
  Synthetic Oligonucleotide
  promoter (1)..(27)
aatttaatacgactcactatagggagagctttcgcagtagttcgtctttaacaaatc

SEQ ID NO: 8 - DNA, 30 bp, Artificial Sequence
  Synthetic Oligonucleotide
gctttcgcagtagttcgtctttaacaaatc

SEQ ID NO: 9 - DNA, 51 bp, Artificial Sequence
  Synthetic Oligonucleotide
aatttaatacgactcactatagggagactttcgcagtagttcgtctttaac

SEQ ID NO: 10 - DNA, 24 bp, Artificial Sequence
  Synthetic Oligonucleotide
ctttcgcagtagttcgtctttaac

SEQ ID NO: 11 - DNA, 20 bp, Artificial Sequence
  Synthetic Oligonucleotide
cttgaatactacagcatgga

SEQ ID NO: 12 - DNA, 20 bp, Artificial Sequence
  Synthetic Oligonucleotide
actacagcatggaataatga

SEQ ID NO: 13 - DNA, 24 bp, Artificial Sequence
  Synthetic Oligonucleotide
cttgaatactacagcatggaataa

SEQ ID NO: 14 - DNA, 20 bp, Artificial Sequence
  Synthetic Oligonucleotide
acttcagcatggaataatga

SEQ ID NO: 15 - DNA, 20 bp, Artificial Sequence
  Synthetic Oligonucleotide
cttgaatacttcagcatgga

SEQ ID NO: 16 - DNA, 20 bp, Artificial Sequence
  Synthetic Oligonucleotide
  variation (4)..(4): "n" means a or g or c or t/u, or unknown, or other (WIPO Standard ST.25 (1998), Appendix 2, Table 1)
  misc_feature (4)..(4): n is a, c, g, or t
actncagcatggaataatga

SEQ ID NO: 17 - DNA, 20 bp, Artificial Sequence
  Synthetic Oligonucleotide
actwcagcatggaataatga

SEQ ID NO: 18 - DNA, 20 bp, Artificial Sequence
  Synthetic Oligonucleotide
  variation (11)..(11): "n" means a or g or c or t/u, or unknown, or other (WIPO Standard ST.25 (1998), Appendix 2, Table 1)
  misc_feature (11)..(11): n is a, c, g, or t
cttgaatactncagcatgga

SEQ ID NO: 19 - DNA, 20 bp, Artificial Sequence
  Synthetic Oligonucleotide
cttgaatactwcagcatgga

SEQ ID NO: 20 - DNA, 20 bp, Artificial Sequence
  Synthetic Oligonucleotide
actttgagaaaactagagtg

SEQ ID NO: 21 - DNA, 20 bp, Artificial Sequence
  Synthetic Oligonucleotide
agaaaactagagtgtttcaa

SEQ ID NO: 22 - DNA, 20 bp, Artificial Sequence
  Synthetic Oligonucleotide
ataatgaagtaggactttgg

SEQ ID NO: 23 - DNA, 20 bp, Artificial Sequence
  Synthetic Oligonucleotide
aggactttggttctattttg

SEQ ID NO: 24 - DNA, 18 bp, Artificial Sequence
  Synthetic Oligonucleotide
ggttctattttgttggtt

SEQ ID NO: 25 - DNA, 17 bp, Artificial Sequence
  Synthetic Oligonucleotide
tggttctattttgttgg

SEQ ID NO: 26 - DNA, 21 bp, Artificial Sequence
  Synthetic Oligonucleotide
ggaataatgaagtaggacttt

SEQ ID NO: 27 - DNA, 20 bp, Artificial Sequence
  Synthetic Oligonucleotide
atggaataatgaagtaggac

SEQ ID NO: 28 - DNA, 18 bp, Artificial Sequence
  Synthetic Oligonucleotide
atggaataatgaagtagg

SEQ ID NO: 29 - DNA, 19 bp, Artificial Sequence
  Synthetic Oligonucleotide
gcatggaataatgaagtag

SEQ ID NO: 30 - DNA, 20 bp, Artificial Sequence
  Synthetic Oligonucleotide
tacagcatggaataatgaag

SEQ ID NO: 31 - DNA, 20 bp, Artificial Sequence
  Synthetic Oligonucleotide
tactacagcatggaataatg

SEQ ID NO: 32 - DNA, 19 bp, Artificial Sequence
  Synthetic Oligonucleotide
agaaaactagagtgtttca

SEQ ID NO: 33 - DNA, 20 bp, Artificial Sequence
  Synthetic Oligonucleotide
agaaaattagagtgtttcaa

SEQ ID NO: 34 - DNA, 21 bp, Artificial Sequence
  Synthetic Oligonucleotide
gagaaaactagagtgtttcaa

SEQ ID NO: 35 - DNA, 21 bp, Artificial Sequence
  Synthetic Oligonucleotide
gagaaaattagagtgtttcaa

SEQ ID NO: 36 - DNA, 20 bp, Artificial Sequence
  Synthetic Oligonucleotide
tgagaaaactagagtgtttc

SEQ ID NO: 37 - DNA, 20 bp, Artificial Sequence
  Synthetic Oligonucleotide
ugaaguaggacuuugguucu

SEQ ID NO: 38 - DNA, 22 bp, Artificial Sequence
  Synthetic Oligonucleotide
uaaugguuaauaggagcaguug

SEQ ID NO: 39 - DNA, 20 bp, Artificial Sequence
  Synthetic Oligonucleotide
aguaaugguuaauaggagca

SEQ ID NO: 40 - DNA, 23 bp, Artificial Sequence
  Synthetic Oligonucleotide
ggacuuugguucuauuuuguugg

SEQ ID NO: 41 - DNA, 25 bp, Artificial Sequence
  Synthetic Oligonucleotide
aaugguuaauaggagcaguuggggg

SEQ ID NO: 42 - DNA, 17 bp, Artificial Sequence
  Synthetic Oligonucleotide
aguaggacuuugguucu

SEQ ID NO: 43 - DNA, 54 bp, Artificial Sequence
  Synthetic Oligonucleotide
  misc_feature (22)..(54): capture sequence
uaggccaauacccuaccgucctttaaaaaaaaaaaaaaaaaaaaaaaaaaaaaa

SEQ ID NO: 44 - DNA, 21 bp, Artificial Sequence
  Synthetic Oligonucleotide
uaggccaauacccuaccgucc

SEQ ID NO: 45 - DNA, 17 bp, Artificial Sequence
  Synthetic Oligonucleotide
atggaataatgaagtag

SEQ ID NO: 46 - DNA, 14 bp, Artificial Sequence
  Synthetic Oligonucleotide
agaaaactagagtg

SEQ ID NO: 47 - DNA, 14 bp, Artificial Sequence
  Synthetic Oligonucleotide
agaaaattagagtg

SEQ ID NO: 48 - DNA, 14 bp, Artificial Sequence
  Synthetic Oligonucleotide
agaaaaytagagtg

SEQ ID NO: 49 - DNA, 18 bp, Artificial Sequence
  Synthetic Oligonucleotide
agaaaactagagtgtttc

SEQ ID NO: 50 - DNA, 18 bp, Artificial Sequence
  Synthetic Oligonucleotide
agaaaattagagtgtttc

SEQ ID NO: 51 - DNA, 18 bp, Artificial Sequence
  Synthetic Oligonucleotide
agaaaaytagagtgtttc

SEQ ID NO: 52 - DNA, 18 bp, Artificial Sequence
  Synthetic Oligonucleotide
tactacagcatggaataa

SEQ ID NO: 53 - DNA, 13 bp, Artificial Sequence
  Synthetic Oligonucleotide
  variation (4)..(4): "n" means a or g or c or t/u, or unknown, or other (WIPO Standard ST.25 (1998), Appendix 2, Table 1)
  misc_feature (4)..(4): n is a, c, g, or t
actncagcatgga

SEQ ID NO: 54 - DNA, 13 bp, Artificial Sequence
  Synthetic Oligonucleotide
actwcagcatgga

SEQ ID NO: 55 - DNA, 13 bp, Artificial Sequence
  Synthetic Oligonucleotide
actacagcatgga

SEQ ID NO: 56 - DNA, 12 bp, Artificial Sequence
  Synthetic Oligonucleotide
gtatttaactgt

SEQ ID NO: 57 - DNA, 22 bp, Artificial Sequence
  Synthetic Oligonucleotide
gtatttaactgtcagaggtgaa

SEQ ID NO: 58 - DNA, 27 bp, Artificial Sequence
  Synthetic Oligonucleotide
aatttaatacgactcactatagggaga

SEQ ID NO: 59 - DNA, 17 bp, Artificial Sequence
  Synthetic Oligonucleotide
aguaggacuuugguucu

SEQ ID NO: 60 - DNA, 18 bp, Artificial Sequence
  Synthetic Oligonucleotide
uaaugguuaauaggagca

SEQ ID NO: 61 - DNA, 1206 bp, Artificial Sequence
  B. microti In Vitro Transcript
gggcgaauuggguaccgggcccccccucgaggucgacgcuuaguauaagcuuuuauacagcgaaacugcgaauggcucauuaaaacaguuauaguuuauuugauguucguuuuacauggauaaccgugguaauucuagggcuaauacaugcucgaggcgcguuuucgcguggcguuuauuagacuuuaaccaacccuucggguaaucggugauucauaauaaauuagcgaaucgcauggcuuugccggcgauguaucauucaaguuucugaccuaucagcuuuggacgguaggguauuggccuaccggggcgacgacgggugacggggaauugggguucgauuccggagagggagccugagaaacggcuaccacaucuaaggaaggcagcaggcgcgcaaauuacccaauccugacacagggagguagugacaagaaauaacaauacagggcuuaaagucuuguaauuggaaugaugggaaucuaaacccuucccagaguaucaauuggagggcaagucuggugccagcagccgcgguaauuccagcuccaauagcguauauuaaaguuguugcaguuaagaagcucguaguugaauuucugccuugucauuaaucucgcuuccgagcguuuuuuuauugacuuggcaucuucuggauuuggugccuucggguacuauuuuccaggauuuacuuugagaaaacuagaguguuucaaacaggcauucgccuugaauacuacagcauggaauaaugaaguaggacuuugguucuauuuuguugguuauugagccagaguaaugguuaauaggagcaguugggggcauucguauuuaacugucagaggugaaauucuuagauuuguuaaagacgaacuacugcgaaagcauuugccaaggauguuuucauuaaucaagaacgaaaguuaggggaucgaagacgaucagauaccgucguaguccuaaccauaaacuaugccgacuagagauuggaggucgucaguuuaaacgacuccuucagcaccuugagagaaaucaaagucuuuggguucuggggggaguauggucgcaagucugaaacuuaaaggaauugacggaagggcaccaccaggcguggagccugcggcuuaauuugacucaacacgggaaaccucaccagguccagacauagagaggauugacagauugauagcucuuucuugaugaauu

SEQ ID NO: 62 - DNA, 1282 bp, Artificial Sequence
  B. divergens In Vitro Transcript
gggcgaauuggguaccgggcccccccucgaggucgacgguaucgauaagcuugauaucgaauuccugcagcccgggggauccaaccugguugauccugccaguagucauaugcuugucuuaaagauuaagccaugcaugucuaaguacaaacuuuuuacggugaaacugcgaauggcucauuacaacaguuauaguuucuuugguauucguuuuccauggauaaccgugcuaauuguagggcuaauacaaguucgaggccuuuuggcggcguuuauuaguucuaaaaccaucccuuuugguuuucggugauucauaauaaacuugcgaaucgcaauuuuuugcgauggaccauucaaguuucugacccaucagcuugacgguaggguauuggccuaccgaggcagcaacggguaacggggaauuaggguucgauuccggagagggagccugagaaacggcuaccacauccaaggaaggcagcaggcgcgcaaauuacccaauccugacacagggagguagugacaagaaauaacaauacagggcaauugucuuguaauuggaaugauggugaccuaaacccucaccagaguaacaauuggagggcaagucuggugccagcagccgcgguaauuccagcuccaauagcguauauuaaacuuguugcaguuaaaaagcucguaguugaauuuuugcgugguguuaauauugacuaaugucgagauugcacuucgcuuuugggauuuaucccuuuuuacuuugagaaaauuagaguguuucaagcagacuuuugucuugaauacuucagcauggaauaauagaguaggacuuugguucuauuuuguugguuugugaaccuuaguaaugguuaauaggaacgguugggggcauucguauuuaacugucagaggugaaauucuuagauuuguuaaagacgaacuacugcgaaagcauuugccaaggacguuuucauuaaucaagaacgaaaguuaggggaucgaagacgaucagauaccgucguaguccuaaccauaaacuaugccgacuagggauuggaggucgucauuuuuccgacuccuucagcaccuugagagaaaucaaagucuuuggguucuggggggaguauggucgcaaggcugaaacuuaaaggaauugacggaagggcaccaccaggcguggagccugcggcuuaauuugacucaacacggggaaacucaccagguccagacaauguuaggauugacagauugauagcucuuucuugauucuuuggguggugcggcc

SEQ ID NO: 63 - DNA, 1251 bp, Artificial Sequence
  B. duncani In Vitro Transcript
gggcgaauuggguaccgggcccccccucgaggucgacguugauccugccaguagucauaugcuugucuuaaagauuaagccaugcaugucuaaguauaaacuuuuauauggugaaacugcgaauggcucauuacaacaguuauaguuuauuugaaagucguuuuuacauggauaaccgugcuaauuguagggcuaauacaugcucgaggccuuggcuccugucuuggcugcguuuauuagacucgaaaccuucccgcuugcgguacucggugauucauaauaaauuugcgaaucgcauggcuuuugccggcgaugguucauucaaguuucugaccuaucagcuuuggacgguaggguauuggccuaccggggcagcgacggguaacggggaauuaggguucgauuccggagagggagccugagaaacggcuaccacaucuaaggaaggcagcaggcgcgcaaauuacccaauacggacaccgugagguagugacaagaaauaacaauacagggcuuaaagcuuuguaauuggaaugaugggaauccaaaccccuuccagaguaucaauuggagggcaagucuggugccagcagccgcgguaauuccagcuccaauagcguauauuaaacuuguugcaguuaaaaagcucguaguugaacuucugccgcuuggccuuucguuccccuugggguuucguucgccugguggcuuaccucuggcggugguucuccauuugccaguuuuacuuugagaaaauuagaguguuucaagcaggcuuuugccuugaauacuucagcauggaauaauaaaguaggacuuugguucuauuuuguugguuucaggaccaaaguaaugguuaauaggaacaguugggggcauucguauuuaacugucagaggugaaauucuuagauuuguuaaagacgaacuacugcgaaagcauuugccaaggauguuuucauuaaucaagaacgaaaguuaggggcucgaagacgaucagauaccgucguaguccuaacuauaaacuaugccgacuagagauuggaggucgucauuuuaaacgacuccuucagcaccuugagagaaaucaaagucuuuggguucuggggggaguauggucgcaaggcugaaacuuaaaggaauugacggaagggcaccaccaggcguggagccugcggcuuaauuugacucaacacggggaaccucaccagguccagacauaguuaggauugacagauugauagcucgaauu

SEQ ID NO: 64 - DNA, 1387 bp, Artificial Sequence
  P. falciparum In Vitro Transcript
gggcgaauuggguaccguagaaacugcgaacggcucauuaaaacaguuauagucuacuugacauuuuuauuauaaggauaacuacggaaaagcuguagcuaauacuugcuuuauuauccuuugauuuuuaucuuuggauaaguauuuguuaggccuuauaagaaaaaaguuauuaacuuaaggaauuauaacaaagaaguaacacguaauaaauuuauuuuauuuaguguguaucaaucgaguuucugaccuaucagcuuuugauguuaggguauuggccuaacauggcuaugacggguaacggggaauuagaguucgauuccggagagggagccugagaaauagcuaccacaucuaaggaaggcagcaggcgcguaaauuacccaauucuaaaaaagagagguagugacaagaaauaacaaugcaaggccaauuuuugguuuuguaauuggaauggugggaauuuaaaaccuucccagaguaacaauuggagggcaagucuggugccagcagccgcgguaauuccagcuccaauagcguauauuaaaauuguugcaguuaaaacgcucguaguugaauuucaaagaaucgauauuuuauuguaacuauucuaggggaacuauuuuagguuuucgcuuuaauacgcuuccucuauuauuauguucuuuaaauaacaaagauucuuuuuaaaauccccacuuuugcuuuuuuggggaauuuguuacuuugaauaaauuagaggugucaaagcaaacaguuaaagcauuuacuguguuugaauacuauagcauggaauaacaaaauugaacaagcuaaaauuuuuuguucuuuuuucuuauuuuggcuuaguuacgauuaauaggaguagcuuggggacauucguauucagaugucagaggugaaauucuuagauuuucuggagacgaacaacugcgaaagcauuugucuaaaauacuuccauuaaucaagaacgaaaguuaagggagugaagacgaucagauaccgucguaaucuuaaccauaaacuaugccgacuagguguuggaugaaaguguuaaaaauaaaagucaucuuucuaggugacuuuuagauugcuuccuucaguaccuuaugagaaaucaaagucuuuggguucuggggcgaguauucgcgcaagcgagaaaguuaaaagaauugacggaagggcaccaccaggcguggagcuugcggcuuaauuugacucaacacggggaaacucacuaguuuaagacaagaguaggauugacagauuaauagcucuuucuugauuucuuggauggugaugcauggccguuuuuaguucgugaauaugauuugucugguuaauuccgauaacgaacgagaucggauccacuaguucuagagcggcc

SEQ ID NO: 65 - DNA, 70 bp, Artificial Sequence
  Synthetic Oligonucleotide
ugaaguaggacuuugguucuauuuuguugguuauugagccagaguaaugguuaauaggagcaguuggggg

SEQ ID NO: 66 - DNA, 34 bp, Artificial Sequence
  Synthetic Oligonucleotide
ttcacctctgacagttaaatacgaatgcccccaa

SEQ ID NO: 67 - DNA, 34 bp, Artificial Sequence
  Synthetic Oligonucleotide
  variation (5)..(5): "n" means a or g or c or t/u, or unknown, or other (WIPO Standard ST.25 (1998), Appendix 2, Table 1)
  misc_feature (5)..(5): n is a, c, g, or t
tactncagcatggaataatgaagtaggactttgg

SEQ ID NO: 68 - DNA, 27 bp, Artificial Sequence
  Synthetic Oligonucleotide
  variation (11)..(11): "n" means a or g or c or t/u, or unknown, or other (WIPO Standard ST.25 (1998), Appendix 2, Table 1)
  misc_feature (11)..(11): n is a, c, g, or t
cttgaatactncagcatggaataatga

SEQ ID NO: 69 - DNA, 11 bp, Artificial Sequence
  Synthetic Oligonucleotide
atggaataatg

SEQ ID NO: 70 - DNA, 27 bp, Artificial Sequence
  Synthetic Oligonucleotide
actttgagaaaaytagagtgtttcaaa

SEQ ID NO: 71 - DNA, 1767 bp, Babesia microti
  ref <308>: AY693840.1
  ref <309>: 2004-09-05
  ref <313>: (1)..(1767)
aacctggttgatcctgccagtagtcatatgcttgtcttaaagattaagccatgcatgtcttagtataagcttttatacagcgaaactgcgaatggctcattaaaacagttatagtttatttgatgttcgttttacatggataaccgtggtaattctagggctaatacatgctcgaggcgcgttttcgcgtggcgtttattagactttaaccaacccttcgggtaatcggtgattcataataaattagcgaatcgcatggctttgccggcgatgtatcattcaagtttctgacctatcagctttggacggtagggtattggcctaccggggcgacgacgggtgacggggaattggggttcgattccggagagggagcctgagaaacggctaccacatctaaggaaggcagcaggcgcgcaaattacccaatcctgacacagggaggtagtgacaagaaataacaatacagggcttaaagtcttgtaattggaatgatgggaatctaaacccttcccagagtatcaattggagggcaagtctggtgccagcagccgcggtaattccagctccaatagcgtatattaaagttgttgcagttaagaagctcgtagttgaatttctgccttgtcattaatctcgcttccgagcgtttttttattgacttggcatcttctggatttggtgccttcgggtactattttccaggatttactttgagaaaactagagtgtttcaaacaggcattcgccttgaatactacagcatggaataatgaagtaggactttggttctattttgttggttattgagccagagtaatggttaataggagcagttgggggcattcgtatttaactgtcagaggtgaaattcttagatttgttaaagacgaactactgcgaaagcatttgccaaggatgttttcattaatcaagaacgaaagttaggggatcgaagacgatcagataccgtcgtagtcctaaccataaactatgccgactagagattggaggtcgtcagtttaaacgactccttcagcaccttgagagaaatcaaagtctttgggttctggggggagtatggtcgcaagtctgaaacttaaaggaattgacggaagggcaccaccaggcgtggagcctgcggcttaatttgactcaacacgggaaacctcaccaggtccagacatagagaggattgacagattgatagctctttcttgattctatgggtggtggtgcatggccgttcttagttggtggagtgatttgtctggttaattccgttaacgaacgagaccttaacctgctaaattaggatctgggacaagctttgctgttccagtatcgcttcttagagggactttgcgttcataaaacgcaaggaagtgtaaggcaataacaggtctgtgatgcccttagatgtcctgggctgcacgcgcgctacactgatgcattcaacgagtttttccttggccgtcgggtccgggtaatcttacagtatgcatcgtgatggggatagattattgcaattattaatcttgaacgaggaatgcctagtaggcgcgagtcatcagctcgtgccgactacgtccctgccctttgtacacaccgcccgtcgctcctaccgatcgagtgatccggtgaattattcggaccaagaaacgtggattcgtccttcgttttttggaaagttttgtgaaccttatcacttaaaggaaggagaagtcgtaacaaggtttccgtaggtgaacctgcggaaggatcattc

SEQ ID NO: 72 - DNA, 1728 bp, Babesia divergens
  ref <308>: AY789076.1
  ref <309>: 2004-11-17
  ref <313>: (1)..(1728)
aacctggttgatcctgccagtagtcatatgcttgtcttaaagattaagccatgcatgtctaagtacaaactttttacggtgaaactgcgaatggctcattacaacagttatagtttctttggtattcgttttccatggataaccgtgctaattgtagggctaatacaagttcgaggccttttggcggcgtttattagttctaaaaccatcccttttggttttcggtgattcataataaacttgcgaatcgcaattttttgcgatggaccattcaagtttctgacccatcagcttgacggtagggtattggcctaccgaggcagcaacgggtaacggggaattagggttcgattccggagagggagcctgagaaacggctaccacatccaaggaaggcagcaggcgcgcaaattacccaatcctgacacagggaggtagtgacaagaaataacaatacagggcaattgtcttgtaattggaatgatggtgacctaaaccctcaccagagtaacaattggagggcaagtctggtgccagcagccgcggtaattccagctccaatagcgtatattaaacttgttgcagttaaaaagctcgtagttgaatttttgcgtggtgttaatattgactaatgtcgagattgcacttcgcttttgggatttatccctttttactttgagaaaattagagtgtttcaagcagacttttgtcttgaatacttcagcatggaataatagagtaggactttggttctattttgttggtttgtgaaccttagtaatggttaataggaacggttgggggcattcgtatttaactgtcagaggtgaaattcttagatttgttaaagacgaactactgcgaaagcatttgccaaggacgttttcattaatcaagaacgaaagttaggggatcgaagacgatcagataccgtcgtagtcctaaccataaactatgccgactagggattggaggtcgtcatttttccgactccttcagcaccttgagagaaatcaaagtctttgggttctggggggagtatggtcgcaaggctgaaacttaaaggaattgacggaagggcaccaccaggcgtggagcctgcggcttaatttgactcaacacggggaaactcaccaggtccagacaatgttaggattgacagattgatagctctttcttgattctttgggtggtggtgcatggccgttcttagttggtggagtgatttgtctggttaattccgttaacgaacgagaccttaacctgctaactagtgtccgtaaaaaggttcgtccgttacggtttgcttcttagagggactttgcggctctaagccgcaaggaagtttaaggcaataacaggtctgtgatgcccttagatgtcctgggctgcacgcgcgctacactgatgcattcatcgagttttatcccttcccgaaagggctgggtaatctttagtatgcatcgtgacggggattgatttttgcaattctaaatcatgaacgaggaatgcctagtatgcgcaagtcatcagcttgtgcagattacgtccctgccctttgtacacaccgcccgtcgctcctaccgatcgagtgatccggtgaattattcggaccgtggcctttccgattcgtcggcttggcctagggaagtcttgtgaaccttatcacttaaaggaaggagaagtcgtaacaaggtttccgtaggtgaacctgcggaaggatcattc

SEQ ID NO: 73 - DNA, 1742 bp, Babesia strain WA1
  ref <308>: AY027815.1
  ref <309>: 2001-03-02
  ref <313>: (1)..(1742)
ccttggttgatcctgccagtagtcatatgcttgtcttaaggattaagccatgcatgtctaagtataaacttttatatggtgaaactgcgaatggctcattacaacagttatagtttatttgaaagtcgtttttacatggataaccgtgctaattgtagggctaatacatgctcgaggccttggcttctgtcttggctgcgtttattagactcgaaaccttcccgcttgcggtactcggtgattcataataaatttgcgaatcgcatggcttttgccggcgatggttcattcaagtttctgacctatcagctttggacggtagggtattggcctaccggggcagcgacgggtaacggggaattagggttcgattccggagagggagcctgagaaacggctaccacatctaaggaaggcagcaggcgcgcaaattacccaatacggacaccgtgaggtagtgacaagaaataacaatacagggctttaagctttgtaattggaatgatgggaatccaaaccccttccagagtatcaattggagggcaagtctggtgccagcagccgcggtaattccagctccaatagcgtatattaaacttgttgcagttaaaaagctcgtagttgaacttctgccgcttggcctttcgttccccttggggtttcgttcgcctggtggcttacctctggcggtggttctccatttgccagttttactttgagaaaattagagtgtttcaagcaggcttttgccttgaatacttcagcatggaataataaagtaggactttggttctattttgttggtttcaggaccaaagtaatggttaataggaacagttgggggcattcgtatttaactgtcagaggtgaaattcttagatttgttaaagacgaactactgcgaaagcatttgccaaggatgttttcattaatcaagaacgaaagttaggggctcgaagacgatcagataccgtcgtagtcctaactataaactatgccgactagagattggaggtcgtcattttaaacgactccttcagcaccttgagagaaatcaaagtctttgggttctggggggagtatggtcgcaaggctgaaacttaaaggaattgacggaagggcaccaccaggcgtggagcctgcggcttaatttgactcaacacggggaacctcaccaggtccagacatagttaggattgacagattgatagctctttcttgattctatgggtagtggtgcatggccgttcttagttggtggagtgatttgtctggttaattccgttaacgaacgagaccttaacctgctaaatagcagctgagaataatctcttgtttcagttttgcttcttagagggactttgcggtcataaatcgcaaggaagtttaaggcaataacaggtctgtgatgcccttagatgtcctgggctgcacgcgcgctacactgatgcattcatcgagttttatccttgcccgaaagggtttggtaatctttagtatgcatcgtgatggggattgattattgcaattattaatcatgaacgaggaatgcctagtaggcgcgagtcatcagctcgtgccgactacgtccctgccctttgtacacaccgcccgtcgctcctaccgatcgagtgatccggtgaattattcggaccgtgacgcttctaattcgttagaaatgtctagggaagttttgtgaaccttatcacttaaaggaaggagaagtcgtaacaaggtttccg

SEQ ID NO: 74 - DNA, 1708 bp, Plasmodium falciparum
  ref <308>: JQ627151.1
  ref <309>: 2012-08-14
  ref <313>: (1)..(1708)
tcaaagattaagccatgcaagtgaaagtatatatatattttatatgtagaaactgcgaacggctcattaaaacagttatagtctacttgacatttttattataaggataactacggaaaagctgtagctaatacttgctttattatcctttgatttttatctttggataagtatttgttaggccttataagaaaaaagttattaacttaaggaattataacaaagaagtaacacgtaataaatttattttatttagtgtgtatcaatcgagtttctgacctatcagcttttgatgttagggtattggcctaacatggctatgacgggtaacggggaattagagttcgattccggagagggagcctgagaaatagctaccacatctaaggaaggcagcaggcgcgtaaattacccaattctaaaaaagagaggtagtgacaagaaataacaatgcaaggccaatttttggttttgtaattggaatggtgggaatttaaaaccttcccagagtaacaattggagggcaagtctggtgccagcagccgcggtaattccagctccaatagcgtatattaaaattgttgcagttaaaacgctcgtagttgaatttcaaagaatcgatattttattgtaactattctaggggaactattttaggttttcgctttaatacgcttcctctattattatgttctttaaataacaaagattctttttaaaatccccacttttgcttttgcttttttggggaatttgttactttgaataaattagaggtgtcaaagcaaacagttaaagcatttactgtgtttgaatactatagcatggaataacaaaattgaacaagctaaaattttttgttcttttttcttattttggcttagttacgattaataggagtagcttggggacattcgtattcagatgtcagaggtgaaattcttagattttctggagacgaacaactgcgaaagcatttgtctaaaatacttccattaatcaagaacgaaagttaagggagtgaagacgatcagataccgtcgtaatcttaaccataaactatgccgactaggtgttggatgaaagtgttaaaaataaaagtcatctttctaggtgacttttagattgcttccttcagtaccttatgagaaatcaaagtctttgggttctggggcgagtattcgcgcaagcgagaaagttaaaagaattgacggaagggcaccaccaggcgtggagcttgcggcttaatttgactcaacacggggaaactcactagtttaagacaagagtaggattgacagattaatagctctttcttgatttcttggatggtgatgcatggccgtttttagttcgtgaatatgatttgtctggttaattccgataacgaacgagatcttaacctgctaattagcggcgagtacactatattcttatttgaaattgaacataggtaactatacatttattcagtaatcaaattaggatatttttattaaaatatccttttccctgttctactaataatttgttttttactctatttctctcttcttttaagaatgtacttgcttgattgaaaagcttcttagaggaacattgtgtgtctaacacaaggaagtttaaggcaacaacaggtctgtgatgtccttagatgaactaggctgcacgcgtgctacactgatatatataacgagtttttaaaaat

SEQ ID NO: 75 - DNA, 23 bp, Artificial Sequence
  Synthetic Oligonucleotide
gaagtaggactttggttctattt

SEQ ID NO: 76 - DNA, 21 bp, Artificial Sequence
  Synthetic Oligonucleotide
atgaagtaggactttggttct

SEQ ID NO: 77 - DNA, 1727 bp, Babesia sp. EU1 venatorum
  ref <308>: AY046575.1
  ref <309>: 2003-07-09
  ref <313>: (1)..(1727)
aacctggttgatcctgccagtagtcatatgcttgtcttaaagattaagccatgcatgtctaagtacaaactttttacggtgaaactgcgaatggctcattacaacagttatagtttctttggtattcgttttccatggataaccgtgctaattgtagggctaatacaagttcgaggccttttggcggcgtttattagttctataaccacccttttggttttcggtgattcataataaactcgcgaatcgcaatttattgcgatggaccattcaagtttctgacccatcagcttgacggtagggtattggcctaccgaggcagcaacgggtaacggggaattagggttcgattccggagagggagcctgagaaacggctaccacatccaaggaaggcagcaggcgcgcaaattacccaatcctgacacagggaggtagtgacaagaaataacaatacagggcaattgtcttgtaattggaatgatggtgacctaaaccctcaccagagtaacaattggagggcaagtctggtgccagcagccgcggtaattccagctccaatagcgtatattaaacttgttgcagttaaaaagctcgtagttgaatttctgcgttatcgagttattgactcttgtctttaatcgatttcgcttttgggatttatccctttttactttgagaaaattagagtgtttcaagcagacttttgtcttgaatacttcagcatggaataatagagtaggactttggttctattttgttggtttttgaaccttagtaatggttaataggaacggttgggggcattcgtatttaactgtcagaggtgaaattcttagatttgttaaagacgaactactgcgaaagcatttgccaaggacgtttccattaatcaagaacgaaagttaggggatcgaagacgatcagataccgtcgtagtcctaaccataaactatgccgactagggattggaggtcgtcatttttccgactccttcagcaccttgagagaaatcaaagtctttgggttctggggggagtatggtcgcaaggctgaaacttaaaggaattgacggaagggcaccaccaggcgtggagcctgcggcttaatttgactcaacacggggaaactcaccaggtccagacaatgttaggattgacagattgatagctctttcttgattctttgggtggtggtgcatggccgttcttagttggtggagtgatttgtctggttaattccgttaacgaacgagaccttaacctgctaactagtacccgtaaaaaggttcgtccgttacggtttgcttcttagagggactttgcggctctaagccgcaaggaagtttaaggcaataacaggtctgtgatgcccttagatgtcctgggctgcacgcgcgctacactgatgcattcatcgagtttaatcctgtcccgaaagggctgggtaatctttagtatgcatcgtgacggggattgatttttgcaattctaaatcatgaacgaggaatgcctagtatgcgcaagtcatcagcttgtgcagattacgtccctgccctttgtacacaccgcccgtcgctcctaccgatcgagtgatccggtgaattattcggaccgtggcttttccgattcgtcggttttgcctagggaagtctcgtgaaccttatcacttaaaggaaggagaagtcgtaacaaggtttccgtaggtgaacctgcagaaggatcaagc

SEQ ID NO: 78 - DNA, 41 bp, Artificial Sequence
  Synthetic Oligonucleotide
gyygccycgguaggccaauacccuaccguccaaagcugaur

SEQ ID NO: 79 - DNA, 41 bp, Artificial Sequence
  Synthetic Oligonucleotide
gyygccycggtaggccaataccctaccgtccaaagctgatr

SEQ ID NO: 80 - DNA, 60 bp, Artificial Sequence
  Synthetic Oligonucleotide
  promoter (1)..(27)
  variation (50)..(50): "n" means a or g or c or t/u, or unknown, or other (WIPO Standard ST.25 (1998), Appendix 2, Table 1)
  misc_feature (50)..(50): n is a, c, g, or t
aatttaatacgactcactatagggagaggcaaatgctttcgcagtagttngtctttaaca

SEQ ID NO: 81 - DNA, 33 bp, Artificial Sequence
  Synthetic oligonucleotide
  variation (23)..(23): "n" means a or g or c or t/u, or unknown, or other (WIPO Standard ST.25 (1998), Appendix 2, Table 1)
  misc_feature (23)..(23): n is a, c, g, or t
ggcaaatgctttcgcagtagttngtctttaaca

SEQ ID NO: 82-83 - skipped (2 entries)

SEQ ID NO: 84 - DNA, 22 bp, Artificial Sequence
  Synthetic oligonucleotide
gcggtaattccagctccaatag

SEQ ID NO: 85 - DNA, 16 bp, Artificial Sequence
  Synthetic oligonucleotide
  variation (11)..(11): "n" means a or g or c or t/u, or unknown, or other (WIPO Standard ST.25 (1998), Appendix 2, Table 1)
  misc_feature (11)..(11): n is a, c, g, or t
cttgaatactncagca

SEQ ID NO: 86 - skipped

SEQ ID NO: 87 - DNA, 56 bp, Artificial Sequence
  Synthetic oligonucleotide
  misc_feature (24)..(56): capture tail
aaagacuuugauuucucucaaggtttaaaaaaaaaaaaaaaaaaaaaaaaaaaaaa

SEQ ID NO: 88 - DNA, 23 bp, Artificial Sequence
  Synthetic oligonucleotide
aaagacuuugauuucucucaagg

SEQ ID NO: 89 - DNA, 61 bp, Artificial Sequence
  Synthetic oligonucleotide
  misc_feature (29)..(61): capture tail
caagaaagagcuaucaaucugucaaucctttaaaaaaaaaaaaaaaaaaaaaaaaaaaaaa

SEQ ID NO: 90 - DNA, 28 bp, Artificial Sequence
  Synthetic oligonucleotide
caagaaagagcuaucaaucugucaaucc

SEQ ID NO: 91 - DNA, 17 bp, Artificial Sequence
  Synthetic oligonucleotide
aguaggacuuugguuct

SEQ ID NO: 92 - DNA, 16 bp, Artificial Sequence
  Synthetic oligonucleotide
aguaggacuuugguuc

SEQ ID NO: 93 - DNA, 17 bp, Artificial Sequence
  Synthetic oligonucleotide
aguaggacuauugguuc

SEQ ID NO: 94 - skipped

SEQ ID NO: 95 - DNA, 95 bp, Artificial Sequence
  Synthetic oligonucleotide
  variation (50)..(50): "n" means a or g or c or t/u, or unknown, or other (WIPO Standard ST.25 (1998), Appendix 2, Table 1)
  misc_feature (50)..(50): n is a, c, g, t or u
actttgagaaaaytagagtgtttcaaacaggccatttgccttgaatactncagcatggaataatgaagtaggactttggttctattttgttggtt

SEQ ID NO: 96 - DNA, 78 bp, Artificial Sequence
  Synthetic oligonucleotide
  variation (23)..(23): "n" means a or g or c or t/u, or unknown, or other (WIPO Standard ST.25 (1998), Appendix 2, Table 1)
  misc_feature (23)..(23): n is a, c, g, t or u
ggcaaatgctttcgcagtagttngtctttaacaaatctaagaatttcacctctgacagttaaatacgaatgcccccaa

SEQ ID NO: 97 - DNA, 37 bp, Artificial Sequence
  Synthetic oligonucleotide
  variation (23)..(23): "n" means a or g or c or t/u, or unknown, or other (WIPO Standard ST.25 (1998), Appendix 2, Table 1)
  misc_feature (23)..(23): n is a, c, g, t or u
ggcaaatgctttcgcagtagttngtctttaacaaatc

SEQ ID NO: 98 - DNA, 18 bp, Artificial Sequence
  Synthetic oligonucleotide
aguaggacuauugguucu

SEQ ID NO: 99 - skipped

SEQ ID NO: 100 - RNA, 1281 nt, Artificial Sequence
  B. venatorum In Vitro Transcript
gggcgaauuggguaccgggcccccccucgaggucgacgguaucgauaagcuugauaucgaauuccugcagcccgggggauccaaccugguugauccugccaguagucauaugcuugucuuaaagauuaagccaugcaugucuaaguacaaacuuuuuacggugaaacugcgaauggcucauuacaacaguuauaguuucuuugguauucguuuuccauggauaaccgugcuaauuguagggcuaauacaaguucgaggccuuuuggcggcguuuauuaguucuauaaccacccuuuugguuuucggugauucauaauaaacucgcgaaucgcaauuuauugcgauggaccauucaaguuucugacccaucagcuugacgguaggguauuggccuaccgaggcagcaacggguaacggggaauuaggguucgauuccggagagggagccugagaaacggcuaccacauccaaggaaggcagcaggcgcgcaaauuacccaauccugacacagggagguagugacaagaaauaacaauacagggcaauugucuuguaauuggaaugauggugaccuaaacccucaccagaguaacaauuggagggcaagucuggugccagcagccgcgguaauuccagcuccaauagcguauauuaaacuuguugcaguuaaaaagcucguaguugaauuucugcguuaucgaguuauugacucuugucuuuaaucgauuucgcuuuugggauuuaucccuuuuuacuuugagaaaauuagaguguuucaagcagacuuuugucuugaauacuucagcauggaauaauagaguaggacuuugguucuauuuuguugguuuuugaaccuuaguaaugguuaauaggaacgguugggggcauucguauuuaacugucagaggugaaauucuuagauuuguuaaagacgaacuacugcgaaagcauuugccaaggacguuuccauuaaucaagaacgaaaguuaggggaucgaagacgaucagauaccgucguaguccuaaccauaaacuaugccgacuagggauuggaggucgucauuuuuccgacuccuucagcaccuugagagaaaucaaagucuuuggguucuggggggaguauggucgcaaggcugaaacuuaaaggaauugacggaagggcaccaccaggcguggagccugcggcuuaauuugacucaacacggggaaacucaccagguccagacaauguuaggauugacagauugauagcucuuucuugauucuuuggguggugcggcc

SEQ ID NO: 101 - DNA, 24 bp, Artificial Sequence
  Synthetic oligonucleotide
  variation (15)..(15): "n" means a or g or c or t/u, or unknown, or other (WIPO Standard ST.25 (1998), Appendix 2, Table 1)
  misc_feature (15)..(15): n is a, c, g, or t
ctttcgcagtagttngtctttaac